European Patent Specification EP 3 921 851 B1, published October 18, 2023. Title: DARC EXPRESSION AS PROGNOSTICATOR OF IMMUNOTHERAPY OUTCOMES. Applicant: CORNELL UNIVERSITY. The sequence listing filed with the application follows.

SEQUENCE LISTING (6 sequences)

SEQ ID NO: 1 - DNA, 30 bp, Homo sapiens
tccttggctcttatcttggaagcacaggcg

SEQ ID NO: 2 - DNA, 30 bp, Homo sapiens
cgcctgtgcttccaagataagagccaagga

SEQ ID NO: 3 - DNA, 20 bp, Artificial Sequence
  primer
tctgggtatgtcctccaggc

SEQ ID NO: 4 - DNA, 20 bp, Artificial Sequence
  primer
aagggcagtgcagagtcatc

SEQ ID NO: 5 - DNA, 20 bp, Artificial Sequence
  primer
tccaatttcccagcacctcc

SEQ ID NO: 6 - DNA, 20 bp, Artificial Sequence
  primer
ggctggttgggactacactc